European Patent Application EP 4 464 713 A1, published November 20, 2024. Title: Circular RNA analogs, preparation and application thereof. Applicant: Sieć Badawcza Łukasiewicz PORT Polski Ośrodek Rozwoju Technologii. The sequence listing filed with the application follows.

SEQUENCE LISTING (12 sequences)

SEQ ID NO: 1 - DNA, 43 bp, synthetic construct
  misc_feature 1..43: note = oligonucleotide ON1
  source 1..43: mol_type = other DNA
agcaaatgtctagattatccctaacatttaaatgcaatgaaaa

SEQ ID NO: 2 - DNA, 10 bp, synthetic construct
  misc_feature 1..10: note = oligonucleotide ON2
  source 1..10: mol_type = other DNA
tccctttttt

SEQ ID NO: 3 - DNA, 28 bp, synthetic construct
  misc_feature 1..28: note = oligonucleotide ON3
  source 1..28: mol_type = other DNA
tctagattatcccttttttttttttttt

SEQ ID NO: 4 - DNA, 48 bp, synthetic construct
  misc_feature 1..48: note = oligonucleotide ON4
  source 1..48: mol_type = other DNA
gaagcaaatgtctagattatcccttttttttttttttttttttttttt

SEQ ID NO: 5 - DNA, 67 bp, synthetic construct
  misc_feature 1..67: note = oligonucleotide ON5
  source 1..67: mol_type = other DNA
gaagcaaatgtctagattatccctttttttttttttttttttttttttttttttgtttaaacattta

SEQ ID NO: 6 - DNA, 51 bp, synthetic construct
  misc_feature 1..51: note = oligonucleotide ON6
  source 1..51: mol_type = other DNA
agggggggagggagaggggtaccccctatccttagtcaccaccggccccct

SEQ ID NO: 7 - DNA, 1332 bp, synthetic construct
  misc_feature 1..1332: note = plasmid PL1
  source 1..1332: mol_type = other DNA
gccgaattatattatttttgccaaataatttttaacaaaagctctgaagtcttcttcatttaaattcttagatgatacttcatctggaaaattgtcccaattagtagcatcacgctgtgtaatacgactcactatagggggtacgccaccatggtgagcaagggcgaggagctgttcaccggggtggtgcccatcctggtcgagctggacggcgacgtaaacggccacaagttcagcgtgtccggcgagggcgagggcgatgccacctacggcaagctgaccctgaagttcatctgcaccaccggcaagctgcccgtgccctggcccaccctcgtgaccaccctgacctacggcgtgcagtgcttcagccgctaccccgaccacatgaagcagcacgacttcttcaagtccgccatgcccgaaggctacgtccaggagcgcaccatcttcttcaaggacgacggcaactacaagacccgcgccgaggtgaagttcgagggcgacaccctggtgaaccgcatcgagctgaagggcatcgacttcaaggaggacggcaacatcctggggcacaagctggagtacaactacaacagccacaacgtctatatcatggccgacaagcagaagaacggcatcaaggtgaacttcaagatccgccacaacatcgaggacggcagcgtgcagctcgccgaccactaccagcagaacacccccatcggcgacggccccgtgctgctgcccgacaaccactacctgagcacccagtccgccctgagcaaagaccccaacgagaagcgcgatcacatggtcctgctggagttcgtgaccgccgccgggatcactctcggcatggacgagctgtacaagtaaggatcctagggccgcagctcgctttcttgctgtccaatttctattaaaggttcctttgttccctaagtccaactactaaactgggggatattatgaagggccttgagcatttggattctgcctaataaaaaacatttattttcattgcgtttagctcgctttcttgctgtccaatttctattaaaggttcctttgttccctaagtccaactactaaactgggggatattatgaagggccttgagcatttggattctgcctaataaaaaacatttattttcattgcatttaaatgtttaaacaaaaaaaaaaaaaaaaaaaaaaaaaaaaaaaaaaaaaaaaaaaaaaaaaaaaaaaaaaaaaaaaaaaaaaaaaaaaaaaaaaaaaaaaaaaaaaaaaaaaaaaaaaaaaaaaaaaaaaaaaaaaaaaagcaggtgggagggtacgttcgtgataaacaaac

SEQ ID NO: 8 - DNA, 1179 bp, synthetic construct
  misc_feature 1..1179: note = plasmid PL2
  source 1..1179: mol_type = other DNA
gcccctgcagccgaattatattatttttgccaaataatttttaacaaaagctctgaagtcttcttcatttaaattcttagatgatacttcatctggaaaattgtcccaattagtagcatcacgctgtgtaatacgactcactatagggggtacgccaccatgggagtcaaagttctgtttgccctgatctgcatcgctgtggccgaggccaagcccaccgagaacaacgaagacttcaacatcgtggccgtggccagcaacttcgcgaccacggatctcgatgctgaccgcgggaagttgcccggcaagaagctgccgctggaggtgctcaaagagttggaagccaatgcccggaaagctggctgcaccaggggctgtctgatctgcctgtcccacatcaagtgcacgcccaagatgaagaagttcatcccaggacgctgccacacctacgaaggcgacaaagagtccgcacagggcggcataggcgaggcgatcgtcgacattcctgagattcctgggttcaaggacttggagcccttggagcagttcatcgcacaggtcgatctgtgtgtggactgcacaactggctgcctcaaagggcttgccaacgtgcagtgttctgacctgctcaagaagtggctgccgcaacgctgtgcgacctttgccagcaagatccagggccaggtggacaagatcaagggggccggtggtgactaaggatcctagggccgcagctcgctttcttgctgtccaatttctattaaaggttcctttgttccctaagtccaactactaaactgggggatattatgaagggccttgagcatttggattctgcctaataaaaaacatttattttcattgcgtttagctcgctttcttgctgtccaatttctattaaaggttcctttgttccctaagtccaactactaaactgggggatattatgaagggccttgagcatttggattctgcctaataaaaaacatttattttcattgcatttaaatgtttaaacaaaaaaaaaaaaaaaaaaaaaaaaaaaaaaaaaaaaaaaaaaaaaaaaaaaaaaaaaaaaaaaaaaaaaaaaaaaaaaaaaaaaaaaaaaaaaaaaaaaaaaaaaaaaaaaaaaaaaaaaaaaaaaaagcaggtgggagggtacgttcgtgataaacaaac

SEQ ID NO: 9 - DNA, 1137 bp, synthetic construct
  misc_feature 1..1137: note = plasmid PL3
  source 1..1137: mol_type = other DNA
ctgcagccgaattatattatttttgccaaataatttttaacaaaagctctgaagtcttcttcatttaaattcttagatgatacttcatctggaaaattgtcccaattagtagcatgccacgctgtgtaatacgactcactatagggataatctagacatttgcttctgacacaactgtgttcactagcaacctcaaacagacaccatgggagtcaaagttctgtttgccctgatctgcatcgctgtggccgaggccaagcccaccgagaacaacgaagacttcaacatcgtggccgtggccagcaacttcgcgaccacggatctcgatgctgaccgcgggaagttgcccggcaagaagctgccgctggaggtgctcaaagagttggaagccaatgcccggaaagctggctgcaccaggggctgtctgatctgcctgtcccacatcaagtgcacgcccaagatgaagaagttcatcccaggacgctgccacacctacgaaggcgacaaagagtccgcacagggcggcataggcgaggcgatcgtcgacattcctgagattcctgggttcaaggacttggagcccttggagcagttcatcgcacaggtcgatctgtgtgtggactgcacaactggctgcctcaaagggcttgccaacgtgcagtgttctgacctgctcaagaagtggctgccgcaacgctgtgcgacctttgccagcaagatccagggccaggtggacaagatcaagggggccggtggtgactaaggatcctagggccgcagctcgctttcttgctgtccaatttctattaaaggttcctttgttccctaagtccaactactaaactgggggatattatgaagggccttgagcatttggattctgcctaataaaaaacatttattttcattgcgtttagctcgctttcttgctgtccaatttctattaaaggttcctttgttccctaagtccaactactaaactgggggatattatgaagggccttgagcatttggattctgcctaataaaaaacatttattttcattgcatttaaatgtttaaacaaaaaaaaaaaaaaaaaaaaaaaaaaaaaaaaaagcaggtgggagggtacgttcgtgataaacaaacggccgc

SEQ ID NO: 10 - DNA, 1667 bp, synthetic construct
  misc_feature 1..1667: note = plasmid PL4
  source 1..1667: mol_type = other DNA
cctgcagccgaattatattatttttgccaaataatttttaacaaaagctctgaagtcttcttcatttaaattcttagatgatacttcatctggaaaattgtcccaattagtagcatgccacgctgtgtaatacgactcactatagggggtacccctctccctccccccctaacgttactggccgaagccgcttggaataaggccggtgtgcgtttgtctatatgttattttccaccatattgccgtcttttggcaatgtgagggcccggaaacctggccctgtcttcttgacgagcattcctaggggtctttcccctctcgccaaaggaatgcaaggtctgttgaatgtcgtgaaggaagcagttcctctggaagcttcttgaagacaaacaacgtctgtagcgaccctttgcaggcagcggaaccccccacctggcgacaggtgcctctgcggccaaaagccacgtgtataagatacacctgcaaaggcggcacaaccccagtgccacgttgtgagttggatagttgtggaaagagtcaaatggctctcctcaagcgtattcaacaaggggctgaaggatgcccagaaggtaccccattgtatgggatctgatctggggcctcggtgcacatgctttacatgtgtttagtcgaggttaaaaaacgtctaggccccccgaaccacggggacgtggttttcctttgaaaaacacgatgataatatggccacacatatgggagtcaaagttctgtttgccctgatctgcatcgctgtggccgaggccaagcccaccgagaacaacgaagacttcaacatcgtggccgtggccagcaacttcgcgaccacggatctcgatgctgaccgcgggaagttgcccggcaagaagctgccgctggaggtgctcaaagagttggaagccaatgcccggaaagctggctgcaccaggggctgtctgatctgcctgtcccacatcaagtgcacgcccaagatgaagaagttcatcccaggacgctgccacacctacgaaggcgacaaagagtccgcacagggcggcataggcgaggcgatcgtcgacattcctgagattcctgggttcaaggacttggagcccttggagcagttcatcgcacaggtcgatctgtgtgtggactgcacaactggctgcctcaaagggcttgccaacgtgcagtgttctgacctgctcaagaagtggctgccgcaacgctgtgcgacctttgccagcaagatccagggccaggtggacaagatcaagggggccggtggtgactaaggatcctagggccgcagctcgctttcttgctgtccaatttctattaaaggttcctttgttccctaagtccaactactaaactgggggatattatgaagggccttgagcatttggattctgcctaataaaaaacatttattttcattgcgtttagctcgctttcttgctgtccaatttctattaaaggttcctttgttccctaagtccaactactaaactgggggatattatgaagggccttgagcatttggattctgcctaataaaaaacatttattttcattgcatttaaatgtttaaacaaaaaaaaaaaaaaaaaaaaaaaaaaaaaaaaaagcaggtgggagggtacgttcgtgataaacaaacggccgct

SEQ ID NO: 11 - DNA, 1111 bp, synthetic construct
  misc_feature 1..1111: note = plasmid PL5
  source 1..1111: mol_type = other DNA
cctgcagccgaattatattatttttgccaaataatttttaacaaaagctctgaagtcttcttcatttaaattcttagatgatacttcatctggaaaattgtcccaattagtagcatgccacgctgtgtaatacgactcactatagggggtaatgagtcctggactgaaacggactcatatgggagtcaaagttctgtttgccctgatctgcatcgctgtggccgaggccaagcccaccgagaacaacgaagacttcaacatcgtggccgtggccagcaacttcgcgaccacggatctcgatgctgaccgcgggaagttgcccggcaagaagctgccgctggaggtgctcaaagagttggaagccaatgcccggaaagctggctgcaccaggggctgtctgatctgcctgtcccacatcaagtgcacgcccaagatgaagaagttcatcccaggacgctgccacacctacgaaggcgacaaagagtccgcacagggcggcataggcgaggcgatcgtcgacattcctgagattcctgggttcaaggacttggagcccttggagcagttcatcgcacaggtcgatctgtgtgtggactgcacaactggctgcctcaaagggcttgccaacgtgcagtgttctgacctgctcaagaagtggctgccgcaacgctgtgcgacctttgccagcaagatccagggccaggtggacaagatcaagggggccggtggtgactaaggatcctagggccgcagctcgctttcttgctgtccaatttctattaaaggttcctttgttccctaagtccaactactaaactgggggatattatgaagggccttgagcatttggattctgcctaataaaaaacatttattttcattgcgtttagctcgctttcttgctgtccaatttctattaaaggttcctttgttccctaagtccaactactaaactgggggatattatgaagggccttgagcatttggattctgcctaataaaaaacatttattttcattgcatttaaatgtttaaacaaaaaaaaaaaaaaaaaaaaaaaaaaaaaaaaaagcaggtgggagggtacgttcgtgataaacaaacggccgct

SEQ ID NO: 12 - DNA, 1287 bp, synthetic construct
  misc_feature 1..1287: note = plasmid PL6
  source 1..1287: mol_type = other DNA
gcccctgcagccgaattatattatttttgccaaataatttttaacaaaagctctgaagtcttcttcatttaaattcttagatgatacttcatctggaaaattgtcccaattagtagcatgccacgctgtgtaatacgactcactatagggggtaggcgcgccagtccttctgtagcgaccctttgcaggcagcggaaccccccacctggcgacaggtgcctctgcggccaaaagccacgtgtataagatacacctgcaaaggcggcacaaccccagtgccacgttgtgagttggatagttgtggaaagagtcaaatggctctcctcaagcgtattcaacaagcgactcggacatatgggagtcaaagttctgtttgccctgatctgcatcgctgtggccgaggccaagcccaccgagaacaacgaagacttcaacatcgtggccgtggccagcaacttcgcgaccacggatctcgatgctgaccgcgggaagttgcccggcaagaagctgccgctggaggtgctcaaagagttggaagccaatgcccggaaagctggctgcaccaggggctgtctgatctgcctgtcccacatcaagtgcacgcccaagatgaagaagttcatcccaggacgctgccacacctacgaaggcgacaaagagtccgcacagggcggcataggcgaggcgatcgtcgacattcctgagattcctgggttcaaggacttggagcccttggagcagttcatcgcacaggtcgatctgtgtgtggactgcacaactggctgcctcaaagggcttgccaacgtgcagtgttctgacctgctcaagaagtggctgccgcaacgctgtgcgacctttgccagcaagatccagggccaggtggacaagatcaagggggccggtggtgactaaggatcctagggccgcagctcgctttcttgctgtccaatttctattaaaggttcctttgttccctaagtccaactactaaactgggggatattatgaagggccttgagcatttggattctgcctaataaaaaacatttattttcattgcgtttagctcgctttcttgctgtccaatttctattaaaggttcctttgttccctaagtccaactactaaactgggggatattatgaagggccttgagcatttggattctgcctaataaaaaacatttattttcattgcatttaaatgtttaaacaaaaaaaaaaaaaaaaaaaaaaaaaaaaaaaaaagcaggtgggagggtacgttcgtgataaacaaacggccgct